European Patent Application EP 4 321 608 A1, published February 14, 2024. Title: Modified filamentous fungus and method of producing proteins using the same. Applicant: Kao Corporation. The sequence listing filed with the application follows.

SEQUENCE LISTING (57 sequences)

SEQ ID NO: 1 - protein, 734 aa, Trichoderma reesei
MATAAAAAAGGAAVAAGADTGAAGSSSTGPPGLPGLPGTRTGSVAMGSAAPAQGSVAAAAGGPPAAGAGAGAVHALTTSPESASASQPGSPTASTTPPQNSLVSAATSFHHHPRGRLVSRACDRCRRRKAKCEYLSAVDSCTHCRDAHVQCTFDLPLARRGPKARKKSDQPGQPPPDPSSLSTAARPGQMPPPLTFSGPAVAALQPFASSSLSPDAAWEPVEPLSIDNGLPRQPLGDLPGLSTIQNISTRQRWIHLANAMTLRNTTLERVSKRCIDLFFDYLYPLTPLVYEPALRDVLAYIFSQPLPGVNQPSPLSQLTPDPTTGTTPLNAAESWAGFGQPSGSRTVGSRLAPWADSTFTLVTAVCAEAAFMLPKDIFPEGESVSEILLEASRDCLHQHLEADLENPTANSIAIRYFHSNCLHAAGKPKYSWHIFGEAIRLAQVMQLHEEAALEGLVPIEAEFRRRCFWILYLGDKSAAILNNRPITIHKYCFDAGITTLYPSGIEDEFLSTASEPPRKSFISGFNANVRLWQSAADLLLEIRVLQDQMMQHFRGTMPPNHVLPSADRQHLDSLYVRFITCLDDLPPYLQSCTLAMAAMAEGNGSAESKQYVIQCINLQVTFHCLRMVITQKFEDLSYFAPGVEQADLRKSEIVRDMLRVMNEAPFWGLQANGEPNVEKIRLIGASLLAIIHRNQDSPLATRARSDFSVLLDILTRLDSKASDQLRNTSTTVVG

SEQ ID NO: 2 - protein, 629 aa, Trichoderma reesei
MLRYSPVLHLDTLSLPPLTNALPRPKCEYLSAVDSCTHCRDAHVQCTFDLPLARRGPKARKKSDQPGQPPPDPSSLSTAARPGQMPPPLTFSGPAVAALQPFASSSLSPDAAWEPVEPLSIDNGLPRQPLGDLPGLSTIQNISTRQRWIHLANAMTLRNTTLERVSKRCIDLFFDYLYPLTPLVYEPALRDVLAYIFSQPLPGVNQPSPLSQLTPDPTTGTTPLNAAESWAGFGQPSGSRTVGSRLAPWADSTFTLVTAVCAEAAFMLPKDIFPEGESVSEILLEASRDCLHQHLEADLENPTANSIAIRYFHSNCLHAAGKPKYSWHIFGEAIRLAQVMQLHEEAALEGLVPIEAEFRRRCFWILYLGDKSAAILNNRPITIHKYCFDAGITTLYPSGIEDEFLSTASEPPRKSFISGFNANVRLWQSAADLLLEIRVLQDQMMQHFRGTMPPNHVLPSADRQHLDSLYVRFITCLDDLPPYLQSCTLAMAAMAEGNGSAESKQYVIQCINLQVTFHCLRMVITQKFEDLSYFAPGVEQADLRKSEIVRDMLRVMNEAPFWGLQANGEPNVEKIRLIGASLLAIIHRNQDSPLATRARSDFSVLLDILTRLDSKASDQLRNTSTTVVG

SEQ ID NO: 3 - protein, 630 aa, Trichoderma atroviride
MLRYAVQYPDTLAISPLTDVFPHQKCEYLSAVDSCTHCRDAHVQCTFDLPLARRGPKARKKSDLPGQPPSDPSALSTGARGAGAQMPPPLAFSGPAVGGLQPFNSSSLSPEAPWEPGEPLSLENGLPRQQMGDLPGLSTIQNISTRQRWLHLAQAMTLRNTTLERVSKRCIDLFFDYLYPLTPLVYEPALREVLAYIFSQPIPGMNQPSPIAQLTPDPTAGTTPLSAAESWAGFAQLNGSRAVGSRLAPWADSTFTLVTAVCAEAAFMLPKDIFPEGESVSEIFLEASRDCLHQHLEADLENPTANSIAIRYFHSNCLHAAGKPKYSWHIFGEAIRLAQVMHLHEEASLEGLVPIEAEFRRRCFWILYLGDKSAAILNNRPITIHKYCFDTGITTLYPSGIEDEFLITASEPPRKSFISGFNANVRLWQSAADLLLEIRVLQDQMMQHFRGNLPPNHVLPSADRQHLDSLYVRFITCLDDLPPYLQSCTLAMAAMAEGNGSAESKQYVIQCTNLQVTFHCLRMVITQKFEDLSYFAPGVEQADLRKSEIVRDMLRVMNEAPFWGLQANGEPNVEKIRLIGASLLAIIHRHQDNPLATRARGDFSVLLDILTRLDSKASDQLRNTSNTVVG

SEQ ID NO: 4 - protein, 630 aa, Trichoderma harzianum
MLRYSSVPSVLQLDPFSSISPLTPHKCEYLSAVDSCTHCRDAHVQCTFDLPLARRGPKARKKSDQPGQPPPDPSSLSTGARGSGQMPPPLSFSGPAAGGLQPFNSSSLSPETAWEPVEPLSIENGLPRQPLGDLPGLSTIQNISTRQRWLHLAHAMTLRSTTLERVSKRCIDLFFDYLYPLTPLVYEPALRDVLAYIFSQPLPGMNQPSPLSQLTPDPTTGTTPISSAESWTGFGQPSGSRIVGSRLAPWVDSTFTLVTAVCAEAAFMLPKDIFPEGESVSEIFLEASRDCLHQHLEADLENPTANSIAIRYFHSNCLHAAGKPKYSWHIFGEAIRLAQVMHLHEEASLEGLVPIEAEFRRRCFWILYLGDKSAAILNNRPITIHKYCFDTGITTLYPSGIEDEFLNTASEPPRKSFISGFNANVRLWQSAADLLLEIRVLQDQMMQHFRGSMPPNHVLPSADRQHLDSLYVRFITCLDDLPPYLQSCTLAMAAMAEGNGSAESKQYVIQCINLQVTFHCLRMVITQKFEDLSYFAPGVEQADLRKSEIVRDMLRVMNEAPFWGLQANGEPNVEKIRLIGASLLAIIHRNQDSPLATRARSDFTVLLDILTRLDSKASDQLRNTSNTVVG

SEQ ID NO: 5 - protein, 940 aa, Trichoderma reesei
MLSNPLRRYSAYPDISSASFDPNYHGSQSHLHSINVNTFGNSHPYPMQHLAQHAELSSSRMIRASPVQPKQRQGSLIAARKNSTGTAGPIRRRISRACDQCNQLRTKCDGLHPCAHCIEFGLGCEYVRERKKRGKASRKDIAAQQAAAAAAQHSGQVQDGPEDQHRKLSRQQSESSRGSAELAQPAHDPPHGHIEGSVSSFSDNGLSQHAAMGGMDGLEDHHGHVGVDPALGRTQLEASSAMGLGAYGEVHPGYESPGMNGHVMVPPSYGAQTTMAGYSGISYAAQAPSPATYSSDGNFRLTGHIHDYPLANGSSPSWGVSLASPSNQFQLQLSQPIFKQSDLRYPVLEPLLPHLGNILPVSLACDLIDLYFSSSSSAQMHPMSPYVLGFVFRKRSFLHPTNPRRCQPALLASMLWVAAQTSEASFLTSLPSARSKVCQKLLELTVGLLQPLIHTGTNSPSPKTSPVVGAAALGVLGVAMPGSLNMDSLAGETGAFGAIGSLDDVITYVHLATVVSASEYKGASLRWWGAAWSLARELKLGRELPPGNPPANQEDGEGLSEDVDEHDLNRNNTRFVTEEEREERRRAWWLVYIVDRHLALCYNRPLFLLDSECSDLYHPMDDIKWQAGKFRSHDAGNSSINIDSSMTDEFGDSPRAARGAHYECRGRSIFGYFLSLMTILGEIVDVHHAKSHPRFGVGFRSARDWDEQVAEITRHLDMYEESLKRFVAKHLPLSSKDKEQHEMHDSGAVTDMQSPLSVRTNASSRMTESEIQASIVVAYSTHVMHVLHILLADKWDPINLLDDDDLWISSEGFVTATSHAVSAAEAISQILEFDPGLEFMPFFYGVYLLQGSFLLLLIADKLQAEASPSVIKACETIVRAHEACVVTLSTEYQRNFSKVMRSALALIRGRVPEDLAEQQQRRRELLALYRWTGNGTGLAL

SEQ ID NO: 6 - DNA, 2918 bp, Trichoderma reesei
atggccacagcggccgcggcagcagctggcggcgcggcggttgctgcgggtgcagacacaggtgcgttgagtcccgtcccgtccgctcgcgttccctcccagctgccagcccgcgtgggtggcactggaacgcagtgcagcgcaatcagtgcagtgcggcccccccaactaacgctgccccccgtggctcctcggccacacaggcgctgcaggctccagctctacaggccctccaggccttccagggcttccaggcacccggacaggctccgtggcgatgggctcagcagctccggcccagggctctgtagctgcagctgcaggcggccctccagctgctggcgctggcgctggcgctgtccacgccctcaccacctcgcccgagtctgcctcggcctcgcagcccggctcgccaaccgcctcaaccacgccgccgcagaactcactcgtgtcggctgcaacctcgttccaccaccatcccagaggccgtctggtgagcagagcctgcgaccgctgccgccggcgcaaggccaaggtcagtctagcccctttgctgttgcttgcatctctgttgtcattgctcctcctcctgctgctgctgatgctgctgctcctcctcctcctcctcctccccgtctcctggtccctggtccctgctcttcatatgtccttactgcccgtgtctcctctccccgttcccgttccccctcctcccgtcctcttctcctgcgtgtctgtcatgcgtacaaagcatacatacaatacatcagcatacatggcaagcgttgtgttgtgttgagagttgtgtgtattgtattgcactgccttcacaactcgttcatactgctgcagcctcaccccaacaccgacctcgtcttccatgctgcgctactcccccgtcttacacctggatactctctccttgccaccactgaccaatgctcttccccgcccaaagtgcgagtacctcagcgctgtcgatagctgcacgcactgccgcgatgcccacgtgcagtgcactttcgacctgcccctggcgcgacgcggccccaaagcgaggaagaagagcgaccagcccggccagccgcctcctgatccgagctcgctctccaccgcggctcgacccggccagatgccgccgccgctgaccttctccggccccgcagtagccgcgctgcagcccttcgcctcgtcgtcgctgtcgcccgacgcggcctgggagcccgtcgagccgctcagcattgacaacggcctgccccggcagccgctgggcgacctgcccggcctctccaccatccagaacatctcgacgcgccagcgatggatacacctggccaacgccatgacgctgcgcaacacgacgctagagcgcgtctcgaagcgatgtatcgacctcttcttcgactacctctaccccctcacccccctggtgtacgagccggccctccgggacgtgctcgcatacatcttctcccagcccttgcctggcgtcaaccaaccatcgccgctgtcacagctcacgccagacccgaccaccggcaccacccccctcaacgctgccgagtcgtgggccggctttggccagcccagcggctcgcgaaccgtcggcagcaggctggctccctgggccgactcgaccttcaccctggtcacggccgtctgcgcagaggcagcattcatgctacccaaggacattttccccgaaggagaatccgtctctgagatcttgctcgaagcctctcgggactgcctgcaccagcacctcgaggccgacctggagaatccgacggccaactcgattgccattcgctacttccactccaactgcctccacgctgcggggaagcccaagtactcgtggcacatatttggcgaggccatccgcctggcgcaggtcatgcagctgcacgaggaggctgccctcgaggggctcgtccccatcgaggcagagttccgccgtcgctgcttttggatcctgtacttgggcgacaagtcagccgctatactcaacaatcggcccatcaccatccacaagtactgcttcgacgccggcatcaccacgctatacccgtcgggtatcgaggacgagttcctgagcacggcgtccgagccgccccggaagagcttcatatccggcttcaacgcaaatgtgcggctctggcagtccgcggctgatttgctgctggaaatccgcgtgctgcaagatcagatgatgcagcactttcgagggaccatgcccccgaaccatgtgctgccctccgccgacaggcagcatctcgattctctctatgtccgcttcatcacctgcttggacgatctcccgccgtacctccagtcgtgcactctggcgatggcagcgatggcagaaggcaacgggtctgccgagtccaagcagtacgtgatacagtgcatcaacctgcaggtgacgtttcactgtctgcgcatggtaattacgcagaaattcgaagacctctcttattttgctcctggcgttgagcaggctgatctcagaaagtcggagattgtgcgagacatgctgagggtgatgaacgaggcgcccttttggggcctgcaggccaatggcgagccaaacgtgagtcgtttccttgtctcttctcttttctgcacacccttttcttcgacgaccccccctctctctttatatccctgcggatatgtatatcatcaagcctcggcacttgttgctaatctgtcctgattatgttgtctggatgctgcaggttgaaaagattcgccttatcggagctagtttgctggccatcatccatcgcaaccaggattcacccttggctacgcgagccaggagcgacttttccgtgcttttggatattctcacgcggctggactcgaaggcgtcggaccaactgaggaatacgtccactaccgttgttggctaa

SEQ ID NO: 7 - DNA, 2038 bp, Trichoderma reesei
atgctgcgctactcccccgtcttacacctggatactctctccttgccaccactgaccaatgctcttccccgcccaaagtgcgagtacctcagcgctgtcgatagctgcacgcactgccgcgatgcccacgtgcagtgcactttcgacctgcccctggcgcgacgcggccccaaagcgaggaagaagagcgaccagcccggccagccgcctcctgatccgagctcgctctccaccgcggctcgacccggccagatgccgccgccgctgaccttctccggccccgcagtagccgcgctgcagcccttcgcctcgtcgtcgctgtcgcccgacgcggcctgggagcccgtcgagccgctcagcattgacaacggcctgccccggcagccgctgggcgacctgcccggcctctccaccatccagaacatctcgacgcgccagcgatggatacacctggccaacgccatgacgctgcgcaacacgacgctagagcgcgtctcgaagcgatgtatcgacctcttcttcgactacctctaccccctcacccccctggtgtacgagccggccctccgggacgtgctcgcatacatcttctcccagcccttgcctggcgtcaaccaaccatcgccgctgtcacagctcacgccagacccgaccaccggcaccacccccctcaacgctgccgagtcgtgggccggctttggccagcccagcggctcgcgaaccgtcggcagcaggctggctccctgggccgactcgaccttcaccctggtcacggccgtctgcgcagaggcagcattcatgctacccaaggacattttccccgaaggagaatccgtctctgagatcttgctcgaagcctctcgggactgcctgcaccagcacctcgaggccgacctggagaatccgacggccaactcgattgccattcgctacttccactccaactgcctccacgctgcggggaagcccaagtactcgtggcacatatttggcgaggccatccgcctggcgcaggtcatgcagctgcacgaggaggctgccctcgaggggctcgtccccatcgaggcagagttccgccgtcgctgcttttggatcctgtacttgggcgacaagtcagccgctatactcaacaatcggcccatcaccatccacaagtactgcttcgacgccggcatcaccacgctatacccgtcgggtatcgaggacgagttcctgagcacggcgtccgagccgccccggaagagcttcatatccggcttcaacgcaaatgtgcggctctggcagtccgcggctgatttgctgctggaaatccgcgtgctgcaagatcagatgatgcagcactttcgagggaccatgcccccgaaccatgtgctgccctccgccgacaggcagcatctcgattctctctatgtccgcttcatcacctgcttggacgatctcccgccgtacctccagtcgtgcactctggcgatggcagcgatggcagaaggcaacgggtctgccgagtccaagcagtacgtgatacagtgcatcaacctgcaggtgacgtttcactgtctgcgcatggtaattacgcagaaattcgaagacctctcttattttgctcctggcgttgagcaggctgatctcagaaagtcggagattgtgcgagacatgctgagggtgatgaacgaggcgcccttttggggcctgcaggccaatggcgagccaaacgtgagtcgtttccttgtctcttctcttttctgcacacccttttcttcgacgaccccccctctctctttatatccctgcggatatgtatatcatcaagcctcggcacttgttgctaatctgtcctgattatgttgtctggatgctgcaggttgaaaagattcgccttatcggagctagtttgctggccatcatccatcgcaaccaggattcacccttggctacgcgagccaggagcgacttttccgtgcttttggatattctcacgcggctggactcgaaggcgtcggaccaactgaggaatacgtccactaccgttgttggctaa

SEQ ID NO: 8 - DNA, 2035 bp, Trichoderma atroviride
atgctgcgctacgccgtccaataccctgatacgctcgcgatctccccactgacagatgttttcccccaccaaaagtgcgaatacctcagcgccgtcgatagctgcacgcactgccgcgatgcacacgtgcagtgcaccttcgacttgccactggcccgacgcggtcccaaagccaggaagaaaagcgatctgcctggccagccaccttcagatccgagcgcgctctccaccggcgcccgtggagccggcgcccagatgccgccgccgttggccttctccggccccgcagtaggtggactgcagcccttcaactcgtcgtcgctgtcgcccgaggctccgtgggagcccggcgagcctctcagcctggagaacgggctgccgcggcagcagatgggcgatctgccgggcctctccaccatccaaaacatctcgacgcgccagcgatggctacacctcgcccaggccatgacgctgcgcaacacgacgctggaacgagtgtcgaagcgatgtatcgacctcttctttgactacctctatcctctcacccccctggtgtacgagccggccctgcgggaggtccttgcatacatcttctcgcagcccatacccggcatgaaccagccctcgcccatcgcgcagctcacgccagacccgacggccgggaccacccccctcagcgctgccgagtcgtgggccggcttcgcgcagctcaatggctcgcgagccgttggcagcaggctggctccctgggccgattcgacctttaccctggtcacagctgtttgcgcagaggcagcatttatgctacccaaagacattttccccgaaggagaatccgtctccgaaatctttcttgaggcttctcgagactgtcttcatcagcatctcgaggccgacctggaaaatccgacggcaaactcaattgccattcggtatttccactccaattgcctccacgccgcggggaaaccaaagtactcgtggcacatctttggcgaggccattcgcctggcccaagttatgcatcttcacgaggaggcgtcgctggaagggcttgtccccattgaggcagagttccgtcggcgctgcttctggattctgtatctgggggacaaatccgcagccatattgaacaaccgtcccataactatccacaaatactgctttgatacgggcatcaccaccctgtacccgtcggggattgaggacgagttcctgattacggcctctgagccgcccaggaagagctttatttccggcttcaacgccaatgtgcggctttggcagtctgcggccgatcttttactggaaatcagggtgctccaagaccagatgatgcaacatttccgcggcaacctgccccccaatcatgtgctgccgtctgcggacaggcagcacctcgactccctctatgttaggttcattacctgtttggacgacctcccgccgtacctccaatcctgcactctggccatggcggccatggccgagggtaacgggtctgcggagtcgaagcagtacgtaattcaatgcacgaatctgcaggtgactttccactgcctgcgcatggtaatcacgcagaagtttgaggatctgtcttactttgctcccggagtagagcaagcagacctgagaaagtcggagattgtgcgagatatgctgagggtgatgaacgaggcgccgttttggggtctccaagcaaacggcgagccaaatgtaagctgctttccttttttcccttgccgtctttccctgcttgcctgtccctctcttctcttctttttttataatgcctgcggtatttatacttttttaagcttcggcatttatatgctaaccttgttatctgatacgacaggttgaaaagatacgccttatcggagctagtttgctagctattatccatcggcatcaggataaccccctggcgacccgagcaaggggcgacttttcagtacttttggatattctgacgcggctagactccaaggcgtctgatcagcttcggaatacttccaataccgttgttggctaa

SEQ ID NO: 9 - DNA, 2012 bp, Trichoderma harzianum
atgctgcgctactcctccgtcccctccgtcttacaacttgatcccttctcctccatctccccactgacaccacacaagtgcgaatacctcagcgccgtcgatagctgcacgcactgccgcgatgcccacgtgcagtgcactttcgacttgccactggcccgacgcggtcccaaagccaggaagaagagcgatcagcccggccagccacctccagacccgagctctctctccaccggggctcgtggatccggccagatgccgccgccgttgagcttctccggccccgcagcaggtggactgcagcccttcaactcgtcctcgctctcgcccgagacggcgtgggagcccgtcgagcctctcagcatcgagaatggcctgccacggcagccgctgggcgacctgcccggcctctccacaattcagaacatctcgactcgccagcggtggctacacctcgcccacgcaatgacgttgcgcagcacgacgctagaacgggtctcgaagcgatgtatcgacctcttcttcgactacctctatcctctcacccccctggtgtacgagcctgccctccgggacgtccttgcatacatcttctcgcagcccttgcccggcatgaaccaaccatcgccgctgtcccagctcacgccagacccgaccactggcaccacccccatcagttctgccgagtcgtggacgggcttcggccagcccagcggctccaggatcgttggcagcaggttggctccttgggtcgactcgaccttcaccctggtcacggccgtctgcgcagaggcagcattcatgctacccaaggacattttccccgaaggagaatccgtctcggaaatctttctcgaggcctctcgcgactgccttcaccagcatctcgaggccgacctggagaatccgacggccaactcgattgccatccgctacttccactccaactgcctccacgccgcggggaagccgaaatactcgtggcacatctttggcgaggccatccgcctggcgcaggtcatgcacctccacgaggaggcttcgctcgaggggctcgtccccatcgaggcagagttccggcgccgttgcttttggattttgtatctgggcgacaagtccgccgctatactcaataaccgtcccatcactatccacaagtactgcttcgacacgggtattactaccctttacccgtctggtattgaggatgagtttctgaacacggcctccgagccgcccagaaaaagctttatttccgggttcaacgcaaacgtgcggctgtggcagtccgccgccgatctgctcctggaaatccgggtgcttcaggaccagatgatgcagcattttaggggcagcatgccccccaaccacgttctgccatctgccgacaggcaacacctcgactccctctatgtcaggttcatcacctgcttggacgacctcccgccgtacctccagtcatgcacgctagccatggcagcaatggccgagggcaacgggtcggccgagtccaagcagtacgtgatccaatgcattaacctgcaggtgacgtttcactgtctgcgcatggtgattacacagaaattcgaagatctctcttattttgctcctggcgttgagcaggccgatttgaggaagtcggagattgtacgagacatgttgagagtgatgaacgaagcgcccttttggggcctccaggccaatggcgagccgaatgtgagtctttttttcttctttgtaattcttctaccgtttctctcttatcaccctgcggatatttatattttaaacttcggcacttgttttgctgaccacttcctatcttgataccgcaggtggaaaagattcgccttatcggagctagtttgttagccattatccatcggaaccaggattcacccctggcgacgcgagctaggagcgactttacggtgctcttggatattctcacgcggctggactccaaggcctcggatcagcttaggaacacgtctaataccgttgttggctaa

SEQ ID NO: 10 - DNA, 2950 bp, Trichoderma reesei
atgttgtccaatcctctccgtcgctattctgcctaccccgacatctcctcggcgtcatttgacccgaactaccatggctcacagtcgcatctccactcgatcaacgtcaacacattcggcaacagccacccctatcccatgcagcacctcgcacagcatgcggagctttcgagttcacgcatgataagggccagtccggtgcagccaaagcagcgccagggctctcttattgctgccaggaagaattcaacgggtactgctgggcccattcggcggaggatcagtcgcgcttgtgaccagtgcaaccagcttcgtaccaagtgcgatggcttacacccatgtgcccattgtataggtatgtcccttttcctctacacagtgatgctgcgctcaagcacatgtactgatcgatcttgtttagaattcggccttggatgcgaatatgtccgagagagaaagaagcgtggcaaagcttcgcgcaaggatattgctgcccagcaagccgcggcggctgcagcacaacactccggccaggtccaggatggtccagaggatcaacatcgcaaactctcacgccagcaaagcgaatcttcgcgtggcagcgctgagcttgcccagcctgcccacgacccgcctcatggccacattgagggctctgtcagctccttcagcgacaatggcctttcccagcatgctgccatgggcggcatggatggcctggaagatcaccatggccacgtcggagttgatcctgccctgggccgaactcagctggaagcgtcatcagcaatgggcctgggcgcatacggtgaagtccaccccggctatgagagccccggcatgaatggccatgtgatggtgcccccgtcgtatggcgcgcagaccaccatggccgggtattccggtatctcgtatgctgcgcaagccccgagtccggctacgtatagcagcgacggtaactttcgactcaccggtcacatccatgattacccgctggcaaatgggagctcgccctcatggggagtctcgctggcctcgccttcgaaccagttccagcttcagctctcgcagcccatcttcaagcaaagcgatttgcgatatcctgtgcttgagcctctgctgcctcacctgggaaacatcctccccgtgtctttggcgtgcgatctgattgacctgtacttctcctcgtcttcatcagcacagatgcacccaatgtccccatacgttctgggcttcgtcttccggaagcgctccttcttgcaccccacgaacccacgaaggtgccagcccgcgctgcttgcgagcatgctgtgggtggcggcacagactagcgaagcgtccttcttgacgagcctgccgtcggcgaggagcaaggtctgccagaagctgctcgagctgaccgttgggcttcttcagcccctgatccacaccggcaccaacagcccgtctcccaagactagccccgtcgtcggtgctgctgccctgggagttcttggggtggccatgccgggctcgctgaacatggattcactggccggcgaaacgggtgcttttggggccatagggagccttgacgacgtcatcacctatgtgcacctcgccacggtcgtctcggccagcgagtacaagggcgccagcctgcggtggtggggtgcggcatggtctctcgccagagagctcaagcttggccgtgagctgccgcctggcaatccacctgccaaccaggaggacggcgagggccttagcgaagacgtggatgagcacgacttgaacagaaacaacactcgcttcgtgacggaagaggagcgcgaagagcgacggcgagcatggtggctcgtttacatcgtcgacaggcacctggcgctctgctacaaccgccccttgtttcttctggacagcgagtgcagcgacttgtaccacccgatggacgacatcaagtggcaggcaggcaaatttcgcagccacgatgcagggaactccagcatcaacatcgatagctccatgacggacgagtttggcgatagtccccgggcggctcgcggcgcacactacgagtgccgcggtcgtagcatttttggctacttcttgtccttgatgacaatcctgggcgagattgtcgatgtccaccatgctaaaagccacccccggttcggcgttggattccgctccgcgcgggattgggacgagcaggttgctgaaatcacccgacacctggacatgtatgaggagagcctcaagaggttcgtggccaagcatctgccattgtcctcaaaggacaaggagcagcatgagatgcacgacagtggagcggtaacagacatgcaatctccactctcggtgcggaccaacgcgtccagccgcatgacggagagcgagatccaggccagcatcgtggtggcttacagcacccatgtgatgcatgtcctccacatcctccttgcggataagtgggatcccatcaaccttctagacgacgacgacttgtggatctcgtcggaaggattcgtgacggcgacgagccacgcggtatcggctgccgaagctattagccagattctcgagtttgaccctggcctggagtttatgccattcttctacggcgtctatctcctgcagggttccttcctcctcctgctcatcgccgacaagctgcaggccgaagcgtctccaagcgtcatcaaggcttgcgagaccattgttagggcacacgaagcttgcgttgtgacgctgagcacagagtatcaggtaagccctatcagttcaaacgtctatcttgctgtgaatcaaagactgacttggacatcagcgcaactttagcaaggttatgcgaagcgcgctggctctgattcggggccgtgtgccggaagatttagctgagcagcagcagcgacgacgcgagcttcttgcactataccgatggactggtaacggaaccggtctggccctctaa

SEQ ID NO: 11 - DNA, 20 bp, Artificial
  Oligonucleotide primer
acggggtacgcgtgaaattg

SEQ ID NO: 12 - DNA, 20 bp, Artificial
  Oligonucleotide primer
tgtgactgattaatgtatga

SEQ ID NO: 13 - DNA, 35 bp, Artificial
  Oligonucleotide primer
taatcagtcacaatggccacagcggccgcggcagc

SEQ ID NO: 14 - DNA, 35 bp, Artificial
  Oligonucleotide primer
tttcgccacggagctttagccaacaacggtagtgg

SEQ ID NO: 15 - DNA, 35 bp, Artificial
  Oligonucleotide primer
cattaatcagtcacaatgctgcgctactcccccgt

SEQ ID NO: 16 - DNA, 35 bp, Artificial
  Oligonucleotide primer
cattaatcagtcacaatgttgtccaatcctctccg

SEQ ID NO: 17 - DNA, 35 bp, Artificial
  Oligonucleotide primer
tttcgccacggagctttagagggccagaccggttc

SEQ ID NO: 18 - DNA, 20 bp, Artificial
  Oligonucleotide primer
agctccgtggcgaaagcctg

SEQ ID NO: 19 - DNA, 20 bp, Artificial
  Oligonucleotide primer
ctcggctacgttgtcatcgt

SEQ ID NO: 20 - DNA, 35 bp, Artificial
  Oligonucleotide primer
gacaacgtagccgagaagtaccgcgcgcttgacaa

SEQ ID NO: 21 - DNA, 35 bp, Artificial
  Oligonucleotide primer
accttggctggtttgctgaatgcccggtggtaagc

SEQ ID NO: 22 - DNA, 20 bp, Artificial
  Oligonucleotide primer
caaaccagccaaggtaggta

SEQ ID NO: 23 - DNA, 35 bp, Artificial
  Oligonucleotide primer
aagcgcgcggtacttccatcacatgtcaatgtcac

SEQ ID NO: 24 - DNA, 20 bp, Artificial
  Oligonucleotide primer
aagtaccgcgcgcttgacaa

SEQ ID NO: 25 - DNA, 20 bp, Artificial
  Oligonucleotide primer
ttggttcttggtttggaggg

SEQ ID NO: 26 - DNA, 35 bp, Artificial
  Oligonucleotide primer
ctagagtatttaaatggtcaacggaggccagaaga

SEQ ID NO: 27 - DNA, 20 bp, Artificial
  Oligonucleotide primer
gactgcctgcctcccagttt

SEQ ID NO: 28 - DNA, 20 bp, Artificial
  Oligonucleotide primer
cataactgagagaaccagaa

SEQ ID NO: 29 - DNA, 35 bp, Artificial
  Oligonucleotide primer
tgcaggtatttaaatattttgcgcatgacgggcga

SEQ ID NO: 30 - DNA, 23 bp, Artificial
  Oligonucleotide primer
atttaaattaacctgatttcaac

SEQ ID NO: 31 - DNA, 20 bp, Artificial
  Oligonucleotide primer
ggcggccgagatctgtgttc

SEQ ID NO: 32 - DNA, 20 bp, Artificial
  Oligonucleotide primer
aaagattgcgacacatacaa

SEQ ID NO: 33 - DNA, 23 bp, Artificial
  Oligonucleotide primer
atttaaatagaggtagtctagtc

SEQ ID NO: 34 - DNA, 35 bp, Artificial
  Oligonucleotide primer
tcacgcgtaccccgtgactgcctgcctcccagttt

SEQ ID NO: 35 - DNA, 35 bp, Artificial
  Oligonucleotide primer
caaaccaagaaccaacataactgagagaaccagaa

SEQ ID NO: 36 - DNA, 35 bp, Artificial
  Oligonucleotide primer
cgccacggagctttagccaacaacggtagtggacg

SEQ ID NO: 37 - DNA, 35 bp, Artificial
  Oligonucleotide primer
caaaccaagaaccaaaaagattgcgacacatacaa

SEQ ID NO: 38 - DNA, 35 bp, Artificial
  Oligonucleotide primer
cagatctcggccgccacggggtacgcgtgaaattg

SEQ ID NO: 39 - DNA, 35 bp, Artificial
  Oligonucleotide primer
taatcagtcacaatgggccccaaagcgaggaagaa

SEQ ID NO: 40 - DNA, 23 bp, Artificial
  Oligonucleotide primer
cattgtgactgattaatgtatga

SEQ ID NO: 41 - DNA, 35 bp, Artificial
  Oligonucleotide primer
taatcagtcacaatggtagccgcgctgcagccctt

SEQ ID NO: 42 - DNA, 35 bp, Artificial
  Oligonucleotide primer
taatcagtcacaatgctctccaccatccagaacat

SEQ ID NO: 43 - DNA, 35 bp, Artificial
  Oligonucleotide primer
taatcagtcacaatgtacctctaccccctcacccc

SEQ ID NO: 44 - DNA, 35 bp, Artificial
  Oligonucleotide primer
taatcagtcacaatgtacatcttctcccagccctt

SEQ ID NO: 45 - DNA, 35 bp, Artificial
  Oligonucleotide primer
cattaatcagtcacaatgctgcgctacgccgtcca

SEQ ID NO: 46 - DNA, 35 bp, Artificial
  Oligonucleotide primer
tttcgccacggagctttagccaacaacggtattgg

SEQ ID NO: 47 - DNA, 35 bp, Artificial
  Oligonucleotide primer
taatcagtcacaatgctgcgctactcctccgtccc

SEQ ID NO: 48 - DNA, 35 bp, Artificial
  Oligonucleotide primer
tttcgccacggagctttagccaacaacggtattag

SEQ ID NO: 49 - DNA, 35 bp, Artificial
  Oligonucleotide primer
taatcagtcacaatgctctccaccatccaaaacat

SEQ ID NO: 50 - DNA, 35 bp, Artificial
  Oligonucleotide primer
taatcagtcacaatgctctccacaattcagaacat

SEQ ID NO: 51 - DNA, 23 bp, Artificial
  Oligonucleotide primer
taaagctccgtggcgaaagcctg

SEQ ID NO: 52 - DNA, 35 bp, Artificial
  Oligonucleotide primer
cgccacggagctttagtccgacgccttcgagtcca

SEQ ID NO: 53 - DNA, 35 bp, Artificial
  Oligonucleotide primer
cgccacggagctttaagccaagggtgaatcctggt

SEQ ID NO: 54 - DNA, 35 bp, Artificial
  Oligonucleotide primer
cgccacggagctttagttcgggggcatggtccctc

SEQ ID NO: 55 - DNA, 35 bp, Artificial
  Oligonucleotide primer
cgccacggagctttatatgaagctcttccggggcg

SEQ ID NO: 56 - DNA, 27 bp, Artificial
  Oligonucleotide primer
cacgcgttctcggctgccgaagctatt

SEQ ID NO: 57 - DNA, 27 bp, Artificial
  Oligonucleotide primer
agccgagaacgcgtggctcgtcgccgt